European Patent Application EP 4 806 919 A1, published September 16, 2026. Title: 抗BCMA单域抗体及其应用. Applicant: 赛斯尔擎生物技术（上海）有限公司. The sequence listing filed with the application follows.

SEQUENCE LISTING (27 sequences)

SEQ ID NO: 1 - protein, 125 aa, Camelus bactrianus
EVQLVQSGGGSVQAGGSLRLSCAASGGDISSTFMGWFRQAPGKEREGVAAIYTGDGTTDYADSVKGRFTIAQDNAKNTVYLEMSRLKPEDTALYYCATGLDGSGSVFSPRSFRYWGQGTQVTVSS

SEQ ID NO: 2 - protein, 7 aa, Camelus bactrianus
GGDISST

SEQ ID NO: 3 - protein, 6 aa, Camelus bactrianus
YTGDGT

SEQ ID NO: 4 - protein, 16 aa, Camelus bactrianus
GLDGSGSVFSPRSFRY

SEQ ID NO: 5 - protein, 5 aa, Camelus bactrianus
STFMG

SEQ ID NO: 6 - protein, 17 aa, Camelus bactrianus
AIYTGDGTTDYADSVKG

SEQ ID NO: 7 - protein, 8 aa, Camelus bactrianus
GGDISSTF

SEQ ID NO: 8 - protein, 8 aa, Camelus bactrianus
IYTGDGTT

SEQ ID NO: 9 - protein, 16 aa, Camelus bactrianus
ATGLDGSGSVFSPRSF

SEQ ID NO: 10 - DNA, 3811 bp, synthetic construct
  source 1..3811: mol_type = other DNA; note = BC-HC-15 CAR-IL15-IL21
cagtttgctttgctgggcctttttcccatgcctgcctttactctgccagagttatattgctggggttttgaagaagatcctattaaataaaagaataagcagtattattaagtagccctgcatttcaggtttccttgagtggcaggccaggcctggccgtgaacgttcactgaaatcatggcctcttggccaagattgatagcttgtgcctgtccctgagtcccagtccatcacgagcagctggtttctaagatgctatttcccgtataaagcatgagaccgtgacttgccagccccacagagccccgcccttgtccatcactggcatctggactccagcctgggttggggcaaagagggaaatgagatcatgtcctaaccctgatcctcttgtcccacattggggttgcgccttttccaaggcagccctgggtttgcgcagggacgcggctgctctgggcgtggttccgggaaacgcagcggcgccgaccctgggtctcgcacattcttcacgtccgttcgcagcgtcacccggatcttcgccgctacccttgtgggccccccggcgacgcttcctgctccgcccctaagtcgggaaggttccttgcggttcgcggcgtgccggacgtgacaaacggaagccgcacgtctcactagtaccctcgcagacggacagcgccagggagcaatggcagcgcgccgaccgcgatgggctgtggccaatagcggctgctcagcagggcgcgccgagagcagcggccgggaaggggcggtgcgggaggcggggtgtggggcggtagtgtgggccctgttcctgcccgcgcggtgttccgcattctgcaagcctccggagcgcacgtcggcagtcggctccctcgttgaccgaatcaccgacctctctccccagggggatcatggccttaccagtgaccgccttgctcctgccgctggccttgctgctccacgccgccaggccggaagtacagctcgtgcagtctgggggaggctcggtgcaggctggagggtctctgagactctcctgcgctgcctctggaggtgatatcagtagcaccttcatgggctggttccgccaggctccaggtaaggagcgcgagggggtcgcagcaatttatactggtgacggcaccaccgactatgccgactccgtgaagggccgattcaccatcgcccaagacaacgccaagaacacggtgtatctcgaaatgagtcgtctgaaacctgaggacactgccttgtactactgtgcgacaggcctggacggcagcggtagcgtcttttcaccccggagctttcgttactggggccaagggacccaggtcaccgtctcctcaaccacgacgccagcgccgcgaccaccaacaccggcgcccaccatcgcgtcgcagcccctgtccctgcgcccagaggcgtgccggccagcggcggggggcgcagtgcacacgagggggctggacttcgcctgtgatatctacatctgggcgcccttggccgggacttgtggggtccttctcctgtcactggttatcaccctttactgcaaacggggcagaaagaaactcctgtatatattcaaacaaccatttatgagaccagtacaaactactcaagaggaagatggctgtagctgccgatttccagaagaagaagaaggaggatgtgaactgagagtgaagttcagcaggagcgcagacgcccccgcgtaccagcagggccagaaccagctctataacgagctcaatctaggacgaagagaggagtacgatgttttggacaagagacgtggccgggaccctgagatggggggaaagccgagaaggaagaaccctcaggaaggcctgtacaatgaactgcagaaagataagatggcggaggcctacagtgagattgggatgaaaggcgagcgccggaggggcaaggggcacgatggcctttaccagggtctcagtacagccaccaaggacacctacgacgcccttcacatgcaggccctgccccctcgcggttctggcgtgaaacagactttgaattttgaccttctcaagttggcgggagacgtggagtccaacccagggcccatgagaatttcgaaaccacatttgagaagtatttccatccagtgctacttgtgtttacttctaaacagtcattttctaactgaagctggcattcatgtcttcattttgggctgtttcagtgcagggcttcctaaaacagaagccaactgggtgaatgtaataagtgatttgaaaaaaattgaagatcttattcaatctatgcatattgatgctactttatatacggaaagtgatgttcaccccagttgcaaagtaacagcaatgaagtgctttctcttggagttacaagttatttcacttgagtccggagatgcaagtattcatgatacagtagaaaatctgatcatcctagcaaacaacagtttgtcttctaatgggaatgtaacagaatctggatgcaaagaatgtgaggaactggaggaaaaaaatattaaagaatttttgcagagttttgtacatattgtccaaatgttcatcaacacttctggaagcggacagtgtactaattatgctctcttgaaattggctggagatgttgagagcaaccctggacctatgagatccagtcctggcaacatggagaggattgtcatctgtctgatggtcatcttcttggggacactggtccacaaatcaagctcccaaggtcaagatcgccacatgattagaatgcgtcaacttatagatattgttgatcagctgaaaaattatgtgaatgacttggtccctgaatttctgccagctccagaagatgtagagacaaactgtgagtggtcagctttttcctgctttcagaaggcccaactaaagtcagcaaatacaggaaacaatgaaaggataatcaatgtatcaattaaaaagctgaagaggaaaccaccttccacaaatgcagggagaagacagaaacacagactaacatgcccttcatgtgattcttatgagaaaaaaccacccaaagaattcctagaaagattcaaatcacttctccaaaagatgattcatcagcatctgtcctctagaacacacggaagtgaagattcctgactgtgccttctagttgccagccatctgttgtttgcccctcccccgtgccttccttgaccctggaaggtgccactcccactgtcctttcctaataaaatgaggaaattgcatcgcattgtctgagtaggtgtcattctattctggggggtggggtggggcaggacagcaagggggaggattgggaagacaatagcaggcatgctggggatgcggtgggctctatgggaattctctagaaatattctcgaggtttaaacgtcgacgcggccgcgatatccagaaccctgaccctgccgtgtaccagctgagagactctaaatccagtgacaagtctgtctgcctattcaccgattttgattctcaaacaaatgtgtcacaaagtaaggattctgatgtgtatatcacagacaaaactgtgctagacatgaggtctatggacttcaagagcaacagtgctgtggcctggagcaacaaatctgactttgcatgtgcaaacgccttcaacaacagcattattccagaagacaccttcttccccagcccaggtaagggcagctttggtgccttcgcaggctgtttccttgcttcaggaatggccaggttctgcccagagctctggtcaatgatgtctaaaactcctctgattggtggtctcggccttatccattgcc

SEQ ID NO: 11 - DNA, 400 bp, synthetic construct
  source 1..400: mol_type = other DNA; note = homologous arm
cagtttgctttgctgggcctttttcccatgcctgcctttactctgccagagttatattgctggggttttgaagaagatcctattaaataaaagaataagcagtattattaagtagccctgcatttcaggtttccttgagtggcaggccaggcctggccgtgaacgttcactgaaatcatggcctcttggccaagattgatagcttgtgcctgtccctgagtcccagtccatcacgagcagctggtttctaagatgctatttcccgtataaagcatgagaccgtgacttgccagccccacagagccccgcccttgtccatcactggcatctggactccagcctgggttggggcaaagagggaaatgagatcatgtcctaaccctgatcctcttgtcccaca

SEQ ID NO: 12 - DNA, 400 bp, synthetic construct
  source 1..400: mol_type = other DNA; note = homologous arm
gatatccagaaccctgaccctgccgtgtaccagctgagagactctaaatccagtgacaagtctgtctgcctattcaccgattttgattctcaaacaaatgtgtcacaaagtaaggattctgatgtgtatatcacagacaaaactgtgctagacatgaggtctatggacttcaagagcaacagtgctgtggcctggagcaacaaatctgactttgcatgtgcaaacgccttcaacaacagcattattccagaagacaccttcttccccagcccaggtaagggcagctttggtgccttcgcaggctgtttccttgcttcaggaatggccaggttctgcccagagctctggtcaatgatgtctaaaactcctctgattggtggtctcggccttatccattgcc

SEQ ID NO: 13 - DNA, 63 bp, synthetic construct
  source 1..63: mol_type = other DNA; note = Signal peptide
atggccttaccagtgaccgccttgctcctgccgctggccttgctgctccacgccgccaggccg

SEQ ID NO: 14 - protein, 21 aa, synthetic construct
  source 1..21: note = Signal peptide
MALPVTALLLPLALLLHAARP

SEQ ID NO: 15 - DNA, 207 bp, synthetic construct
  source 1..207: mol_type = other DNA; note = Hinge-TM domain
accacgacgccagcgccgcgaccaccaacaccggcgcccaccatcgcgtcgcagcccctgtccctgcgcccagaggcgtgccggccagcggcggggggcgcagtgcacacgagggggctggacttcgcctgtgatatctacatctgggcgcccttggccgggacttgtggggtccttctcctgtcactggttatcaccctttactgc

SEQ ID NO: 16 - protein, 69 aa, synthetic construct
  source 1..69: note = Hinge-TM domain
TTTPAPRPPTPAPTIASQPLSLRPEACRPAAGGAVHTRGLDFACDIYIWAPLAGTCGVLLLSLVITLYC

SEQ ID NO: 17 - DNA, 462 bp, synthetic construct
  source 1..462: mol_type = other DNA; note = 41BBz
aaacggggcagaaagaaactcctgtatatattcaaacaaccatttatgagaccagtacaaactactcaagaggaagatggctgtagctgccgatttccagaagaagaagaaggaggatgtgaactgagagtgaagttcagcaggagcgcagacgcccccgcgtaccagcagggccagaaccagctctataacgagctcaatctaggacgaagagaggagtacgatgttttggacaagagacgtggccgggaccctgagatggggggaaagccgagaaggaagaaccctcaggaaggcctgtacaatgaactgcagaaagataagatggcggaggcctacagtgagattgggatgaaaggcgagcgccggaggggcaaggggcacgatggcctttaccagggtctcagtacagccaccaaggacacctacgacgcccttcacatgcaggccctgccccctcgc

SEQ ID NO: 18 - protein, 154 aa, synthetic construct
  source 1..154: note = 41BBz
KRGRKKLLYIFKQPFMRPVQTTQEEDGCSCRFPEEEEGGCELRVKFSRSADAPAYQQGQNQLYNELNLGRREEYDVLDKRRGRDPEMGGKPRRKNPQEGLYNELQKDKMAEAYSEIGMKGERRRGKGHDGLYQGLSTATKDTYDALHMQALPPR

SEQ ID NO: 19 - DNA, 489 bp, synthetic construct
  source 1..489: mol_type = other DNA; note = IL-15
atgagaatttcgaaaccacatttgagaagtatttccatccagtgctacttgtgtttacttctaaacagtcattttctaactgaagctggcattcatgtcttcattttgggctgtttcagtgcagggcttcctaaaacagaagccaactgggtgaatgtaataagtgatttgaaaaaaattgaagatcttattcaatctatgcatattgatgctactttatatacggaaagtgatgttcaccccagttgcaaagtaacagcaatgaagtgctttctcttggagttacaagttatttcacttgagtccggagatgcaagtattcatgatacagtagaaaatctgatcatcctagcaaacaacagtttgtcttctaatgggaatgtaacagaatctggatgcaaagaatgtgaggaactggaggaaaaaaatattaaagaatttttgcagagttttgtacatattgtccaaatgttcatcaacacttcttga

SEQ ID NO: 20 - protein, 162 aa, synthetic construct
  source 1..162: note = IL-15
MRISKPHLRSISIQCYLCLLLNSHFLTEAGIHVFILGCFSAGLPKTEANWVNVISDLKKIEDLIQSMHIDATLYTESDVHPSCKVTAMKCFLLELQVISLESGDASIHDTVENLIILANNSLSSNGNVTESGCKECEELEEKNIKEFLQSFVHIVQMFINTS

SEQ ID NO: 21 - DNA, 489 bp, synthetic construct
  source 1..489: mol_type = other DNA; note = IL-21
atgagatccagtcctggcaacatggagaggattgtcatctgtctgatggtcatcttcttggggacactggtccacaaatcaagctcccaaggtcaagatcgccacatgattagaatgcgtcaacttatagatattgttgatcagctgaaaaattatgtgaatgacttggtccctgaatttctgccagctccagaagatgtagagacaaactgtgagtggtcagctttttcctgctttcagaaggcccaactaaagtcagcaaatacaggaaacaatgaaaggataatcaatgtatcaattaaaaagctgaagaggaaaccaccttccacaaatgcagggagaagacagaaacacagactaacatgcccttcatgtgattcttatgagaaaaaaccacccaaagaattcctagaaagattcaaatcacttctccaaaagatgattcatcagcatctgtcctctagaacacacggaagtgaagattcctga

SEQ ID NO: 22 - protein, 162 aa, synthetic construct
  source 1..162: note = IL-21
MRSSPGNMERIVICLMVIFLGTLVHKSSSQGQDRHMIRMRQLIDIVDQLKNYVNDLVPEFLPAPEDVETNCEWSAFSCFQKAQLKSANTGNNERIINVSIKKLKRKPPSTNAGRRQKHRLTCPSCDSYEKKPPKEFLERFKSLLQKMIHQHLSSRTHGSEDS

SEQ ID NO: 23 - DNA, 514 bp, synthetic construct
  source 1..514: mol_type = other DNA; note = PGK promoter
ttggggttgcgccttttccaaggcagccctgggtttgcgcagggacgcggctgctctgggcgtggttccgggaaacgcagcggcgccgaccctgggtctcgcacattcttcacgtccgttcgcagcgtcacccggatcttcgccgctacccttgtgggccccccggcgacgcttcctgctccgcccctaagtcgggaaggttccttgcggttcgcggcgtgccggacgtgacaaacggaagccgcacgtctcactagtaccctcgcagacggacagcgccagggagcaatggcagcgcgccgaccgcgatgggctgtggccaatagcggctgctcagcagggcgcgccgagagcagcggccgggaaggggcggtgcgggaggcggggtgtggggcggtagtgtgggccctgttcctgcccgcgcggtgttccgcattctgcaagcctccggagcgcacgtcggcagtcggctccctcgttgaccgaatcaccgacctctctccccagggggatc

SEQ ID NO: 24 - DNA, 1044 bp, synthetic construct
  source 1..1044: mol_type = other DNA; note = BC-HC-15 CAR
gaagtacagctcgtgcagtctgggggaggctcggtgcaggctggagggtctctgagactctcctgcgctgcctctggaggtgatatcagtagcaccttcatgggctggttccgccaggctccaggtaaggagcgcgagggggtcgcagcaatttatactggtgacggcaccaccgactatgccgactccgtgaagggccgattcaccatcgcccaagacaacgccaagaacacggtgtatctcgaaatgagtcgtctgaaacctgaggacactgccttgtactactgtgcgacaggcctggacggcagcggtagcgtcttttcaccccggagctttcgttactggggccaagggacccaggtcaccgtctcctcaaccacgacgccagcgccgcgaccaccaacaccggcgcccaccatcgcgtcgcagcccctgtccctgcgcccagaggcgtgccggccagcggcggggggcgcagtgcacacgagggggctggacttcgcctgtgatatctacatctgggcgcccttggccgggacttgtggggtccttctcctgtcactggttatcaccctttactgcaaacggggcagaaagaaactcctgtatatattcaaacaaccatttatgagaccagtacaaactactcaagaggaagatggctgtagctgccgatttccagaagaagaagaaggaggatgtgaactgagagtgaagttcagcaggagcgcagacgcccccgcgtaccagcagggccagaaccagctctataacgagctcaatctaggacgaagagaggagtacgatgttttggacaagagacgtggccgggaccctgagatggggggaaagccgagaaggaagaaccctcaggaaggcctgtacaatgaactgcagaaagataagatggcggaggcctacagtgagattgggatgaaaggcgagcgccggaggggcaaggggcacgatggcctttaccagggtctcagtacagccaccaaggacacctacgacgcccttcacatgcaggccctgccccctcgc

SEQ ID NO: 25 - protein, 348 aa, synthetic construct
  source 1..348: note = BC-HC-15 CAR
EVQLVQSGGGSVQAGGSLRLSCAASGGDISSTFMGWFRQAPGKEREGVAAIYTGDGTTDYADSVKGRFTIAQDNAKNTVYLEMSRLKPEDTALYYCATGLDGSGSVFSPRSFRYWGQGTQVTVSSTTTPAPRPPTPAPTIASQPLSLRPEACRPAAGGAVHTRGLDFACDIYIWAPLAGTCGVLLLSLVITLYCKRGRKKLLYIFKQPFMRPVQTTQEEDGCSCRFPEEEEGGCELRVKFSRSADAPAYQQGQNQLYNELNLGRREEYDVLDKRRGRDPEMGGKPRRKNPQEGLYNELQKDKMAEAYSEIGMKGERRRGKGHDGLYQGLSTATKDTYDALHMQALPPR

SEQ ID NO: 26 - DNA, 1179 bp, synthetic construct
  source 1..1179: mol_type = other DNA; note = EF1a promoter
ggctccggtgcccgtcagtgggcagagcgcacatcgcccacagtccccgagaagttggggggaggggtcggcaattgaaccggtgcctagagaaggtggcgcggggtaaactgggaaagtgatgtcgtgtactggctccgcctttttcccgagggtgggggagaaccgtatataagtgcagtagtcgccgtgaacgttctttttcgcaacgggtttgccgccagaacacaggtaagtgccgtgtgtggttcccgcgggcctggcctctttacgggttatggcccttgcgtgccttgaattacttccacctggctgcagtacgtgattcttgatcccgagcttcgggttggaagtgggtgggagagttcgaggccttgcgcttaaggagccccttcgcctcgtgcttgagttgaggcctggcctgggcgctggggccgccgcgtgcgaatctggtggcaccttcgcgcctgtctcgctgctttcgataagtctctagccatttaaaatttttgatgacctgctgcgacgctttttttctggcaagatagtcttgtaaatgcgggccaagatctgcacactggtatttcggtttttggggccgcgggcggcgacggggcccgtgcgtcccagcgcacatgttcggcgaggcggggcctgcgagcgcggccaccgagaatcggacgggggtagtctcaagctggccggcctgctctggtgcctggcctcgcgccgccgtgtatcgccccgccctgggcggcaaggctggcccggtcggcaccagttgcgtgagcggaaagatggccgcttcccggccctgctgcagggagctcaaaatggaggacgcggcgctcgggagagcgggcgggtgagtcacccacacaaaggaaaagggcctttccgtcctcagccgtcgcttcatgtgactccacggagtaccgggcgccgtccaggcacctcgattagttctcgagcttttggagtacgtcgtctttaggttggggggaggggttttatgcgatggagtttccccacactgagtgggtggagactgaagttaggccagcttggcacttgatgtaattctccttggaatttgccctttttgagtttggatcttggttcattctcaagcctcagacagtggttcaaagtttttttcttccatttcaggtgtcgtga

SEQ ID NO: 27 - DNA, 20 bp, synthetic construct
  source 1..20: mol_type = other DNA; note = sgRNA
tcagggttctggatatctgt